European Patent Specification EP 4 153 212 B1, published October 15, 2025. Title: PEPTIDE FOR USE IN THE PREVENTION AND/OR TREATMENT OF A DISEASE CAUSED BY A VIRUS AFFECTING THE RESPIRATORY TRACT. Applicant: Fundacion para el Fomento de la Investigacion Sanitaria y Biomedica de la Comunitat Valenciana (FISABIO). The sequence listing filed with the application follows.

SEQUENCE LISTING (32 sequences)

SEQ ID NO: 1 - protein, 42 aa, other sequences
  LEK-42
LEKGLDGAKKAVGGLGKLGKDAVEDLESVGKGAVHDVKDVLD

SEQ ID NO: 2 - protein, 45 aa, other sequences
  LEK-45
LEKGLDGAKKAVGGLGKLGKDAVEDLESVGKGAVHDVKDVLDSVL

SEQ ID NO: 3 - protein, 45 aa, other sequences
  SSL-45
SSLLEKGLDGAKKAVGGLGKLGKDAVEDLESVGKGAVHDVKDVLD

SEQ ID NO: 4 - protein, 47 aa, other sequences
  DCD
SSLLEKGLDGAKKAVGGLGKLGKDAVEDLESVGKGAVHDVKDVLDSV

SEQ ID NO: 5 - protein, 48 aa, other sequences
  DCD-1L
SSLLEKGLDGAKKAVGGLGKLGKDAVEDLESVGKGAVHDVKDVLDSVL

SEQ ID NO: 6 - protein, 46 aa, other sequences
  SSL-46
SSLLEKGLDGAKKAVGGLGKLGKDAVEDLESVGKGAVHDVKDVLDS

SEQ ID NO: 7 - protein, 44 aa, other sequences
  LEK-44
LEKGLDGAKKAVGGLGKLGKDAVEDLESVGKGAVHDVKDVLDSV

SEQ ID NO: 8 - protein, 43 aa, other sequences
  LEK-43
LEKGLDGAKKAVGGLGKLGKDAVEDLESVGKGAVHDVKDVLDS

SEQ ID NO: 9 - protein, 28 aa, other sequences
  SSL-29
SSLLEKGDGAKKAVGGLGKLGKDAVEDL

SEQ ID NO: 10 - protein, 25 aa, other sequences
  SSL-25
SSLLEKGLDGAKKAVGGLGKLGKDA

SEQ ID NO: 11 - protein, 41 aa, other sequences
  LEK-41
LEKGLDGAKKAVGGLGKLGKDAVEDLESVGKGAVHDVKDVL

SEQ ID NO: 12 - protein, 26 aa, other sequences
  LEK-26
LEKGLDGAKKAVGGLGKLGKDAVEDL

SEQ ID NO: 13 - protein, 24 aa, other sequences
  LEK-24
LEKGLDGAKKAVGGLGKLGKDAVE

SEQ ID NO: 14 - protein, 42 aa, other sequences
  YDP-42
YDPEAASAPGSGNPCHEASAAQKENAGEDPGLARQAPKPRKQ

SEQ ID NO: 15 - protein, 30 aa, other sequences
  Y-P30
YDPEAASAPGSGNPCHEASAAQKENAGEDP

SEQ ID NO: 16 - protein, 20 aa, other sequences
  PIF
YDPEAASAPGSGNPCHEASA

SEQ ID NO: 17 - protein, 110 aa, other sequences
  Dermcidin
MRFMTLLFLTALAGALVCAYDPEAASAPGSGNPCHEASAAQKENAGEDPGLARQAPKPRKQRSSLLEKGLDGAKKAVGGLGKLGKDAVEDLESVGKGAVHDVKDVLDSVL

SEQ ID NO: 18 - protein, 20 aa, other sequences
  EB_FGF-4 signal sequence
RRKKAAVALLPAVLLALLAP

SEQ ID NO: 19 - protein, 42 aa, other sequences; identical to SEQ ID NO: 1
  LEK-42
  MOD_RES 3: ACETYLATION

SEQ ID NO: 20 - protein, 45 aa, other sequences; identical to SEQ ID NO: 2
  LEK-45
  MOD_RES 3: ACETYLATION

SEQ ID NO: 21 - protein, 45 aa, other sequences; identical to SEQ ID NO: 3
  SSL-45
  MOD_RES 6: ACETYLATION

SEQ ID NO: 22 - protein, 47 aa, other sequences; identical to SEQ ID NO: 4
  DCD
  MOD_RES 6: ACETYLATION

SEQ ID NO: 23 - protein, 48 aa, other sequences; identical to SEQ ID NO: 5
  DCD-1L
  MOD_RES 6: ACETYLATION

SEQ ID NO: 24 - protein, 46 aa, other sequences; identical to SEQ ID NO: 6
  SSL-46
  MOD_RES 6: ACETYLATION

SEQ ID NO: 25 - protein, 44 aa, other sequences; identical to SEQ ID NO: 7
  LEK-44
  MOD_RES 3: ACETYLATION

SEQ ID NO: 26 - protein, 43 aa, other sequences; identical to SEQ ID NO: 8
  LEK-43
  MOD_RES 3: ACETYLATION

SEQ ID NO: 27 - protein, 28 aa, other sequences
  SSL-29
  MOD_RES 6: ACETYLATION
SSLLEKGDGAKKAVGGLGKLGKDAVEDL

SEQ ID NO: 28 - protein, 25 aa, other sequences
  SSL-25
  MOD_RES 6: ACETYLATION
SSLLEKGLDGAKKAVGGLGKLGKDA

SEQ ID NO: 29 - protein, 41 aa, other sequences; identical to SEQ ID NO: 11
  LEK-41
  MOD_RES 3: ACETYLATION

SEQ ID NO: 30 - protein, 26 aa, other sequences
  LEK-26
  MOD_RES 3: ACETYLATION
LEKGLDGAKKAVGGLGKLGKDAVEDL

SEQ ID NO: 31 - protein, 24 aa, other sequences
  LEK-24
  MOD_RES 3: ACETYLATION
LEKGLDGAKKAVGGLGKLGKDAVE

SEQ ID NO: 32 - protein, 110 aa, other sequences; identical to SEQ ID NO: 17
  Dermcidin
  MOD_RES 68: ACETYLATION